European Patent Application EP 4 176 934 A1, published May 10, 2023. Title: Lipidized cocaine- and amphetamine-regulated transcript peptide analogues as anti-obesity and neuroprotective agents. Applicant: Ustav organicke chemie a biochemie AV CR, v. v. i. Application EP. The sequence listing filed with the application follows.

SEQUENCE LISTING (7 sequences)

SEQ ID NO: 1 - protein, 42 aa, synthetic construct
  REGION 1..42: note = modified CARTp
  LIPID 1: note = C8-C16 acyl
  MOD_RES 7: note = Nle
  DISULFID 14..34: note = disulfide bridge
  DISULFID 28..41: note = disulfide bridge
KYGQVPXADAGEQCAVRKGARIGKLADCPRGTSCNSFLLKCL

SEQ ID NO: 2 - protein, 42 aa, synthetic construct; identical to SEQ ID NO: 1
  REGION 1..42: note = modified CARTp
  LIPID 1: note = octanoyl
  MOD_RES 7: note = Nle
  DISULFID 14..34: note = disulfide bridge
  DISULFID 28..41: note = disulfide bridge

SEQ ID NO: 3 - protein, 42 aa, synthetic construct; identical to SEQ ID NO: 1
  REGION 1..42: note = modified CARTp
  LIPID 1: note = myristoyl
  MOD_RES 7: note = Nle
  DISULFID 14..34: note = disulfide bridge
  DISULFID 28..41: note = disulfide bridge

SEQ ID NO: 4 - protein, 42 aa, synthetic construct; identical to SEQ ID NO: 1
  REGION 1..42: note = modified CARTp
  LIPID 1: note = palmitoyl
  MOD_RES 7: note = Nle
  DISULFID 14..34: note = disulfide bridge
  DISULFID 28..41: note = disulfide bridge

SEQ ID NO: 5 - protein, 42 aa, synthetic construct
  REGION 1..42: note = CART(61-102)
  DISULFID 8..26: note = disulfide bridge
  DISULFID 14..34: note = disulfide bridge
  DISULFID 28..41: note = disulfide bridge
KYGQVPMCDAGEQCAVRKGARIGKLCDCPRGTSCNSFLLKCL

SEQ ID NO: 6 - protein, 42 aa, synthetic construct; identical to SEQ ID NO: 1
  REGION 1..42: note = modified CARTp
  MOD_RES 7: note = Nle
  DISULFID 14..34: note = disulfide bridge
  DISULFID 28..41: note = disulfide bridge

SEQ ID NO: 7 - protein, 42 aa, synthetic construct
  REGION 1..42: note = modified CARTp
  LIPID 1: note = palmitoyl
  MOD_RES 7: note = Nle
  DISULFID 14..34: note = disulfide bridge
  DISULFID 26..41: note = disulfide bridge
KYGQVPXADAGEQCAVRKGARIGKLCDAPRGTSCNSFLLKCL